European Patent Application EP 4 365 597 A2, published May 8, 2024. Title: Methods of Assaying Proteins. Applicant: Nautilus Subsidary, INC. The sequence listing filed with the application follows.

SEQUENCE LISTING (15 sequences)

SEQ ID NO: 1 - protein, 30 aa, synthetic construct
  REGION 1..30: note = Description of Artificial Sequence: Synthetic polypeptide
MKLTLKNLSMAIMMSIVMGSSAMAADSNEK

SEQ ID NO: 2 - protein, 8 aa, synthetic construct
  REGION 1..8: note = Description of Artificial Sequence: Synthetic peptide
GYLPEHTL

SEQ ID NO: 3 - protein, 7 aa, synthetic construct
  REGION 1..7: note = Description of Artificial Sequence: Synthetic peptide
ADYLEQD

SEQ ID NO: 4 - protein, 5 aa, synthetic construct
  REGION 1..5: note = Description of Artificial Sequence: Synthetic peptide
TYPGR

SEQ ID NO: 5 - protein, 7 aa, synthetic construct
  REGION 1..7: note = Description of Artificial Sequence: Synthetic peptide
LHDHYLD

SEQ ID NO: 6 - protein, 7 aa, synthetic construct
  REGION 1..7: note = Description of Artificial Sequence: Synthetic peptide
DRARKDG

SEQ ID NO: 7 - protein, 5 aa, synthetic construct
  REGION 1..5: note = Description of Artificial Sequence: Synthetic peptide
TFEEE

SEQ ID NO: 8 - protein, 8 aa, synthetic construct
  REGION 1..8: note = Description of Artificial Sequence: Synthetic peptide
DEIKSLKF

SEQ ID NO: 9 - protein, 10 aa, synthetic construct
  REGION 1..10: note = Description of Artificial Sequence: Synthetic peptide
QTYPGRFPMG

SEQ ID NO: 10 - protein, 18 aa, synthetic construct
  REGION 1..18: note = Description of Artificial Sequence: Synthetic peptide
HTFEEEIEFVQGLNHSTG

SEQ ID NO: 11 - protein, 40 aa, synthetic construct
  REGION 1..40: note = Description of Artificial Sequence: Synthetic polypeptide
NIGIYPEIKAPWFHQEGKDIAAKTLEVLKKYGYTGKDDKV

SEQ ID NO: 12 - protein, 244 aa, Aequorea victoria
MSKGEELFTGVVPILVELDGDVNGHKFSVSGEGEGDATYGKLTLKFICTTGKLPVPWPTLVTTFSYGVQCFSRYPDHMKQHDFFKSAMPEGYVQERTIFFKDDGNYKTRAEVKFEGDTLVNRIELKGIDFKEDGNILGHKLEYNYNSHNVYIMADKQKNGIKVNFKIRHNIEDGSVQLADHYQQNTPIGDGPVLLPDNHYLSTQSALSKDPNEKRDHMVLLEFVTAAGITHGMDELYKHHHHHH

SEQ ID NO: 13 - protein, 150 aa, Bos taurus
MALKSLVLLSLLVLVLLLVRVQPSLGKETAAAKFERQHMDSSTSAASSSNYCNQMMKSRNLTKDRCKPVNTFVHESLADVQAVCSQKNVACKNGQTNCYQSYSTMSITDCRETGSSKYPNCAYKTTQANKHIIVACEGNPYVPVHFDASV

SEQ ID NO: 14 - protein, 710 aa, Homo sapiens
MKLVFLVLLFLGALGLCLAGRRRSVQWCAVSQPEATKCFQWQRNMRKVRGPPVSCIKRDSPIQCIQAIAENRADAVTLDGGFIYEAGLAPYKLRPVAAEVYGTERQPRTHYYAVAVVKKGGSFQLNELQGLKSCHTGLRRTAGWNVPIGTLRPFLNWTGPPEPIEAAVARFFSASCVPGADKGQFPNLCRLCAGTGENKCAFSSQEPYFSYSGAFKCLRDGAGDVAFIRESTVFEDLSDEAERDEYELLCPDNTRKPVDKFKDCHLARVPSHAVVARSVNGKEDAIWNLLRQAQEKFGKDKSPKFQLFGSPSGQKDLLFKDSAIGFSRVPPRIDSGLYLGSGYFTAIQNLRKSEEEVAARRARVVWCAVGEQELRKCNQWSGLSEGSVTCSSASTTEDCIALVLKGEADAMSLDGGYVYTAGKCGLVPVLAENYKSQQSSDPDPNCVDRPVEGYLAVAVVRRSDTSLTWNSVKGKKSCHTAVDRTAGWNIPMGLLFNQTGSCKFDEYFSQSCAPGSDPRSNLCALCIGDEQGENKCVPNSNERYYGYTGAFRCLAENAGDVAFVKDVTVLQNTDGNNNEAWAKDLKLADFALLCLDGKRKPVTEARSCHLAMAPNHAVVSRMDKVERLKQVLLHQQAKFGRNGSDCPDKFCLFQSETKNLLFNDNTECLARLHGKTTYEKYLGPQYVAGITNLKKCSTSPLLEACEFLRK

SEQ ID NO: 15 - protein, 243 aa, Schistosoma japonicum
STMSPILGYWKIKGLVQPTRLLLEYLEEKYEEHLYERDEGDKWRNKKFELGLEFPNLPYYIDGDVKLTQSMAIIRYIADKHNMLGGCPKERAEISMLEGAVLDIRYCVSRIAYSKDFETLKVDFLSKLPEMLKMFEDRLCHKTYLNGDHVTHPDFMLYDALDVVLYMDPMCLDAFPKLVCFKKRIEAIPQIDKYLKSSKYIAWPLQGWQATFGGGDHPPKSDLVPRGSPLEVLFQGPCGSYGS